European Patent Specification EP 3 600 398 B1, published September 13, 2023. Title: HUMAN PD1 PEPTIDE VACCINES AND USES THEREOF. Applicant: Ohio State Innovation Foundation. The sequence listing filed with the application follows.

SEQUENCE LISTING (30 sequences)

SEQ ID NO: 1 - protein, 126 aa, Artificial Sequence
  synthetic construct
PPTFSPALLVVTEGDNATFTCSFSNTSESFVLNWYRMSPSNQTDKLAAFPEDRSQPGQDCRFRVTQLPNGRDFHMSVVRARRNDSGTYLCGAISLAPKLQIKESLRAERVTERRAEVPTAHPSPSP

SEQ ID NO: 2 - protein, 19 aa, Artificial Sequence
  synthetic construct
VLNWYRMSPSNQTDKLAAF

SEQ ID NO: 3 - protein, 19 aa, Artificial Sequence
  synthetic construct
KLAAFPEDRSQPGQDCRFR

SEQ ID NO: 4 - protein, 18 aa, Artificial Sequence
  synthetic construct
DFHMSVVRARRNDSGTYL

SEQ ID NO: 5 - protein, 19 aa, Artificial Sequence
  synthetic construct
GAISLAPKAQIKESLRAEL

SEQ ID NO: 6 - protein, 18 aa, Artificial Sequence
  synthetic construct
KLLSLIKGVIVHRLEGVE

SEQ ID NO: 7 - protein, 4 aa, Artificial Sequence
  synthetic construct
GPSL

SEQ ID NO: 8 - protein, 41 aa, Artificial Sequence
  synthetic construct
KLLSLIKGVIVHRLEGVEGPSLVLNWYRMSPSNQTDKLAAF

SEQ ID NO: 9 - protein, 41 aa, Artificial Sequence
  synthetic construct
KLLSLIKGVIVHRLEGVEGPSLKLAAFPEDRSQPGQDCRFR

SEQ ID NO: 10 - protein, 40 aa, Artificial Sequence
  synthetic construct
KLLSLIKGVIVHRLEGVEGPSLDFHMSVVRARRNDSGTYL

SEQ ID NO: 11 - protein, 41 aa, Artificial Sequence
  synthetic construct
KLLSLIKGVIVHRLEGVEGPSLGAISLAPKAQIKESLRAEL

SEQ ID NO: 12 - protein, 19 aa, Artificial Sequence
  synthetic construct
FAALKDTQNSPSMRYWNLV

SEQ ID NO: 13 - protein, 19 aa, Artificial Sequence
  synthetic construct
RFRCDQGPQSRDEPFAALK

SEQ ID NO: 14 - protein, 18 aa, Artificial Sequence
  synthetic construct
LYTGSDNRRARVVSMHFD

SEQ ID NO: 15 - protein, 19 aa, Artificial Sequence
  synthetic construct
LEARLSEKIQAKPALSIAG

SEQ ID NO: 16 - protein, 41 aa, Artificial Sequence
  synthetic construct
KLLSLIKGVIVHRLEGVEGPSLFAALKDTQNSPSMRYWNLV

SEQ ID NO: 17 - protein, 41 aa, Artificial Sequence
  synthetic construct
KLLSLIKGVIVHRLEGVEGPSLRFRCDQGPQSRDEPFAALK

SEQ ID NO: 18 - protein, 40 aa, Artificial Sequence
  synthetic construct
KLLSLIKGVIVHRLEGVEGPSLLYTGSDNRRARVVSMHFD

SEQ ID NO: 19 - protein, 41 aa, Artificial Sequence
  synthetic construct
KLLSLIKGVIVHRLEGVEGPSLLEARLSEKIQAKPALSIAG

SEQ ID NO: 20 - protein, 19 aa, Artificial Sequence
  synthetic construct
NSVDDALINSTIYSYFPSV

SEQ ID NO: 21 - protein, 17 aa, Artificial Sequence
  synthetic construct
PGINGKAIHLVNNQSSE

SEQ ID NO: 22 - protein, 15 aa, Artificial Sequence
  synthetic construct
QYIKANSKFIGITEL

SEQ ID NO: 23 - protein, 21 aa, Artificial Sequence
  synthetic construct
FNNFTVSFWLRVPKVSASHLE

SEQ ID NO: 24 - protein, 15 aa, Artificial Sequence
  synthetic construct
LSEIKGVIVHRLEGV

SEQ ID NO: 25 - protein, 15 aa, Artificial Sequence
  synthetic construct
FFLLTRILTIPQSLN

SEQ ID NO: 26 - protein, 20 aa, Artificial Sequence
  synthetic construct
TCGVGVRVRSRVNAANKKPE

SEQ ID NO: 27 - protein, 31 aa, Artificial Sequence
  synthetic construct
LHCPALVTYNTDTFESMPNPEGRYTFGASCV

SEQ ID NO: 28 - protein, 53 aa, Artificial Sequence
  synthetic construct
KLLSLIKGVIVHRLEGVEGPSLLHCPALVTYNTDTFESMPNPEGRYTFGASCV

SEQ ID NO: 29 - protein, 30 aa, Artificial Sequence
  synthetic construct
VARCPSGVKPDLSYMPIWKFPDEEGACQPL

SEQ ID NO: 30 - protein, 52 aa, Artificial Sequence
  synthetic construct
KLLSLIKGVIVHRLEGVEGPSLVARCPSGVKPDLSYMPIWKFPDEEGACQPL